European Patent Specification EP 3 580 235 B1, published May 1, 2024. Title: NEUTRALIZING ANTIBODIES TO PLASMODIUM FALCIPARUM CIRCUMSPOROZOITE PROTEIN AND THEIR USE. Applicant: The United States of America, as Represented by the Secretary, Department of Health and Human SErvices. The sequence listing filed with the application follows.

SEQUENCE LISTING (124 sequences)

SEQ ID NO: 1 - protein, 121 aa, homo sapiens
QVQLVQSGAEVKKPGASVKVSCKASGYTFTSYAIHWVRQAPGQRLEWMGWIKAGNGDTRYSQKFQGRVTITRDTSATTAYMELSSLRSEDTAVYYCGLLTVLTPDDAFDIWGQGTMVTVSS

SEQ ID NO: 2 - protein, 113 aa, homo sapiens
DIVMTQSPDSLAVSLGERATINCKSSQSVLYSSNNKNYLAWYQQKPGQPPKLLIYWASIRESGVPDRFSGSGSGTDFTLTISSLQAEDVAVYYCHQYYSSPLTFGGGTKVEIK

SEQ ID NO: 3 - protein, 121 aa, homo sapiens
QVQLVQSGPEVKKPGTSVKVSCKASGFTFSSSAVQWVRQARGQRLEWIGWIVVGSGKTKYAQNFQQRVTITRDMSTSTAYLELSTLRSEDTAVYYCAAVVNWNDESGFDPWGQGTLVTVSS

SEQ ID NO: 4 - protein, 106 aa, homo sapiens
DIQMTQSPSSLSAFVGDRVTITCRASQSIGTYLNWYQQKVGQAPKLLIYTASSLRSGVPSRFSGSGSGTDFTLTITSLQPEDFATYYCQQSYSTYTFGQGTKLEIK

SEQ ID NO: 5 - protein, 122 aa, homo sapiens
EVQLVESGGGVVQPGRSLRLSCAASGFTFSSYGMYWVRQAPGKGLEWVALISHDGSNKFYADSVKGRFTISRDNSKNTLYLQMNSLRAEDTAVYYCAKDLGYSSSWGYFDYWGQGTLVTVSS

SEQ ID NO: 6 - protein, 106 aa, homo sapiens
EIVLTQSPATLSLSPGERATLSCRASQSVSSYLAWYQQKPGQAPRLLIYDASNRATGIPARFSGSGSGTDFTLTISSLEPEDFAVYYCQQRSNWYTFGQGTKLEIK

SEQ ID NO: 7 - protein, 124 aa, homo sapiens
QVQLVESGGGVVQPGRSLRLSCAASGFTFSSYGIHWVRQAPGKGLEWVAVIWYDGSKKYYGDSVKGRFTISRDNSKNTLYLQMNSLRVEDTAVYYCARAVIAATGTRGYWFDPWGQGTLVTVSS

SEQ ID NO: 8 - protein, 106 aa, homo sapiens
DIIMTQSPVSLSASVGDRVTITCRASQSISSHLNWYQQKPGKAPKLLIYAASSLQSGVPSRFSGSGSGTDFTLTISSLQPEDFATYSCQQTYRGFTFAPGTKVDIK

SEQ ID NO: 9 - protein, 119 aa, homo sapiens
QVQLVQSGSELKKPGASVKVSCKTSGYTFTTYAMNWVRQAPGQGLEWMGWINTNTGNPTYAPGFTGRFVFSFDTSVSTAYLQISSLKAEDTAVYYCARVYSYGVPFDYWGQGTLVTVSS

SEQ ID NO: 10 - protein, 110 aa, homo sapiens
QSVLTQPASVSGSPGQSITISCTATSSNVGSFNLVSWYQHHPGKAPKLIIHEVSKRPSGASNRFSGSKSGNTASLTISGLQAEDEADYYCCSYVGSDTWVFGGGTKLTVL

SEQ ID NO: 11 - protein, 121 aa, homo sapiens
QVQLVQSGAEVKKPGASVKVSCKASGYTFTSYAIHWVRQAPGQRLEWMGWIKAGNGNTRYSQKFQDRVTITRDTSTTTAYMELSSLRSEDTAVYYCALLTVLTPDDAFDIWGQGTMVTVSS

SEQ ID NO: 12 - protein, 113 aa, homo sapiens
DIVMTQSPDSLAVSLGERATINCKSSQSVLYSSNNKNYLAWYQQKPGQPPNLLIYWASTRQSGVPDRFSGSGSGTDFTLTISSLQAEDVAVYYCHQYYSSPLTFGGGTKVEIK

SEQ ID NO: 13 - protein, 451 aa, homo sapiens
QVQLVQSGAEVKKPGASVKVSCKASGYTFTSYAIHWVRQAPGQRLEWMGWIKAGNGNTRYSQKFQDRVTITRDTSTTTAYMELSSLRSEDTAVYYCALLTVLTPDDAFDIWGQGTMVTVSSASTKGPSVFPLAPSSKSTSGGTAALGCLVKDYFPEPVTVSWNSGALTSGVHTFPAVLQSSGLYSLSSVVTVPSSSLGTQTYICNVNHKPSNTKVDKKVEPKSCDKTHTCPPCPAPELLGGPSVFLFPPKPKDTLMISRTPEVTCVVVDVSHEDPEVKFNWYVDGVEVHNAKTKPREEQYNSTYRVVSVLTVLHQDWLNGKEYKCKVSNKALPAPIEKTISKAKGQPREPQVYTLPPSRDELTKNQVSLTCLVKGFYPSDIAVEWESNGQPENNYKTTPPVLDSDGSFFLYSKLTVDKSRWQQGNVFSCSVMHEALHNHYTQKSLSLSPGK

SEQ ID NO: 14 - protein, 220 aa, homo sapiens
DIVMTQSPDSLAVSLGERATINCKSSQSVLYSSNNKNYLAWYQQKPGQPPNLLIYWASTRQSGVPDRFSGSGSGTDFTLTISSLQAEDVAVYYCHQYYSSPLTFGGGTKVEIKRTVAAPSVFIFPPSDEQLKSGTASVVCLLNNFYPREAKVQWKVDNALQSGNSQESVTEQDSKDSTYSLSSTLTLSKADYEKHKVYACEVTHQGLSSPVTKSFNRGEC

SEQ ID NO: 15 - protein, 4 aa, homo sapiens
YAIH

SEQ ID NO: 16 - protein, 17 aa, homo sapiens
WIKAGNGDTRYSQKFQG

SEQ ID NO: 17 - protein, 13 aa, homo sapiens
LLTVLTPDDAFDI

SEQ ID NO: 18 - protein, 17 aa, homo sapiens
KSSQSVLYSSNNKNYLA

SEQ ID NO: 19 - protein, 7 aa, homo sapiens
WASIRES

SEQ ID NO: 20 - protein, 9 aa, homo sapiens
HQYYSSPLT

SEQ ID NO: 21 - protein, 4 aa, homo sapiens
SAVQ

SEQ ID NO: 22 - protein, 17 aa, homo sapiens
WIVVGSGKTKYAQNFQQ

SEQ ID NO: 23 - protein, 13 aa, homo sapiens
AVVNWNDESGFDP

SEQ ID NO: 24 - protein, 11 aa, homo sapiens
RASQSIGTYLN

SEQ ID NO: 25 - protein, 7 aa, homo sapiens
TASSLRS

SEQ ID NO: 26 - protein, 8 aa, homo sapiens
QQSYSTYT

SEQ ID NO: 27 - protein, 4 aa, homo sapiens
YGMY

SEQ ID NO: 28 - protein, 17 aa, homo sapiens
LISHDGSNKFYADSVKG

SEQ ID NO: 29 - protein, 14 aa, homo sapiens
KDLGYSSSWGYFDY

SEQ ID NO: 30 - protein, 11 aa, homo sapiens
RASQSVSSYLA

SEQ ID NO: 31 - protein, 7 aa, homo sapiens
DASNRAT

SEQ ID NO: 32 - protein, 8 aa, homo sapiens
QQRSNWYT

SEQ ID NO: 33 - protein, 4 aa, homo sapiens
YGIH

SEQ ID NO: 34 - protein, 17 aa, homo sapiens
VIWYDGSKKYYGDSVKG

SEQ ID NO: 35 - protein, 16 aa, homo sapiens
RAVIAATGTRGYWFDP

SEQ ID NO: 36 - protein, 11 aa, homo sapiens
RASQSISSHLN

SEQ ID NO: 37 - protein, 7 aa, homo sapiens
AASSLQS

SEQ ID NO: 38 - protein, 8 aa, homo sapiens
QQTYRGFT

SEQ ID NO: 39 - protein, 4 aa, homo sapiens
YAMN

SEQ ID NO: 40 - protein, 17 aa, homo sapiens
WINTNTGNPTYAPGFTG

SEQ ID NO: 41 - protein, 11 aa, homo sapiens
RVYSYGVPFDY

SEQ ID NO: 42 - protein, 14 aa, homo sapiens
TATSSNVGSFNLVS

SEQ ID NO: 43 - protein, 7 aa, homo sapiens
EVSKRPS

SEQ ID NO: 44 - protein, 10 aa, homo sapiens
CSYVGSDTWV

SEQ ID NO: 45 - protein, 17 aa, homo sapiens
WIKAGNGNTRYSQKFQD

SEQ ID NO: 46 - protein, 7 aa, homo sapiens
WASTRQS

SEQ ID NO: 47 - DNA, 363 bp, homo sapiens
caggtgcagcttgtgcagtctggggctgaggtgaagaagcctggggcctcagtgaaggtttcctgcaaggcctctggatacaccttcactagttatgctatacattgggtgcgccaggcccccggacaaaggcttgagtggatgggatggatcaaggctggcaatggtgatacaagatattcacagaagttccagggcagagtcaccattaccagggacacatccgcgaccacagcctacatggagctgagcagcctgagatctgaagacacggctgtatattactgtggcctacttacggtgctaactcctgatgatgcatttgatatctggggccaagggacaatggtcaccgtctcttca

SEQ ID NO: 48 - DNA, 339 bp, homo sapiens
gacatcgtgatgacccagtctccagactccctggctgtgtctctgggcgagagggccaccatcaactgcaagtccagccagagtgttttatacagctccaacaataagaactacttagcttggtaccagcagaaaccaggacagcctcctaagctgctcatttattgggcatctatccgggaatccggggtccctgaccgattcagtggcagcgggtctgggacagatttcactctcaccatcagcagcctgcaggctgaagatgtggcagtttattactgtcaccagtattatagtagtcctctcactttcggcggagggaccaaggtggaaatcaaa

SEQ ID NO: 49 - DNA, 363 bp, homo sapiens
caggtgcagctggtgcagtctgggcctgaggtgaagaagcctgggacctcagtgaaggtctcctgcaaggcttctggattcacctttagtagctctgctgtgcagtgggtgcgacaggctcgtggacaacgccttgagtggataggatggatcgtcgttggcagtggtaagacaaagtacgcacagaacttccaacaaagagtcaccattaccagggacatgtccacaagtacagcctatctggagctgagcaccctgagatccgaggacacggccgtgtattactgtgcggcagttgtcaactggaacgacgaaagcgggttcgacccctggggccagggaaccctggtcaccgtctcctca

SEQ ID NO: 50 - DNA, 318 bp, homo sapiens
gacatccagatgacccagtctccatcgtccctgtctgcatttgtgggagacagagtcaccatcacttgccgggcaagtcagagcattggcacctatttaaattggtatcagcagaaagtaggtcaagcccctaagctcctgatatatactgcatccagtctgcgaagtggggtcccatcaaggttcagtggcagtggatctgggacagatttcactctcaccatcaccagtctgcaacctgaagattttgcaacttactactgtcaacagagttacagtacctacacttttggccaggggaccaagctggagatcaaa

SEQ ID NO: 51 - DNA, 366 bp, homo sapiens
gaggtgcagttggtggagtctgggggaggcgtggtccagcctgggaggtccctgagactctcctgtgcagcctctggattcaccttcagtagctatggcatgtactgggtccgccaggctccaggcaaggggctggagtgggtggcacttatatcacatgatggaagtaataaattctatgcagactccgtgaagggccgattcaccatctccagagacaattccaagaacacgctgtatctgcaaatgaacagcctgagagctgaggacacggctgtgtattactgtgcgaaagacttgggttatagcagcagctgggggtactttgactactggggccagggaaccctggtcaccgtctcctca

SEQ ID NO: 52 - DNA, 318 bp, homo sapiens
gaaattgtgttgacacagtctccagccaccctgtctttgtctccaggggaaagagccaccctctcctgcagggccagtcagagtgttagcagctacttagcctggtaccaacagaaacctggccaggctcccaggctcctcatctatgatgcatccaacagggccactggcatcccagccaggttcagtggcagtgggtctgggacagacttcactctcaccatcagcagcctagagcctgaagattttgcagtttattactgtcagcagcgtagcaactggtacacttttggccaggggaccaagctggagatcaaa

SEQ ID NO: 53 - DNA, 372 bp, homo sapiens
caggtgcagctggtggagtctgggggaggcgtggtccagcctgggaggtccctgagactctcctgtgcagcgtctggattcaccttcagtagctatggcatacactgggtccgccaggctccaggcaaggggctggagtgggtggcagttatatggtatgatggaagtaagaaatattatggagactctgtgaagggccgattcaccatctccagagacaattccaagaacacgctgtatctgcaaatgaacagcctgagagtcgaggacacggctgtgtattactgtgcgagggctgttatagcagcaactggtacgcgaggttactggttcgacccctggggccagggaaccctggtcaccgtctcctca

SEQ ID NO: 54 - DNA, 318 bp, homo sapiens
gacatcattatgacccagtctccagtctccctgtctgcatctgtaggagacagagtcaccatcacttgccgggcaagtcagagcattagcagccatttaaattggtatcagcagaaaccagggaaagcccctaagctcctgatctatgctgcatccagtttgcaaagtggggtcccatcaaggttcagtggcagtggatctgggacagatttcactctcaccatcagcagtctgcaacctgaagattttgcaacttactcctgtcaacagacttacagggggttcactttcgcccctgggaccaaagtggatatcaaa

SEQ ID NO: 55 - DNA, 357 bp, homo sapiens
caggtgcagctggtgcaatctgggtctgagttgaagaagcctggggcctcagtgaaggtttcctgcaagacttctggatacaccttcactacctatgctatgaattgggtgcgacaggcccctggacaagggcttgagtggatgggatggatcaacaccaacactggaaacccaacgtacgccccgggcttcacagggcggtttgtcttctccttcgacacctctgtcagcacggcatatctgcagatcagcagcctgaaggctgaggacactgccgtttattactgtgcgagagtctacagctatggggtcccatttgactactggggccagggaaccctggtcaccgtctcctca

SEQ ID NO: 56 - DNA, 371 bp, homo sapiens
cagtctgtgctgactcagcctgcctccgtgtctgggtctcctggacagtcgatcaccatctcctgcactgcaaccagcagtaatgttgggagttttaaccttgtctcctggtaccaacatcacccaggcaaagcccccaaactcatcattcatgaggtcagtaagcggccctcaggggcttctaatcgcttctctggctccaagtctggcaacacggcctccctgacaatctctgggctccaggctgaggacgaggctgattattactgctgctcatatgtaggcagtgacacttgggtgttcggcggagggaccaagctgaccgtcctgggtcagcccaaggctgccccctcggtcactctgttcccgcc

SEQ ID NO: 57 - DNA, 363 bp, homo sapiens
caggtgcagcttgtgcagtctggggctgaggtgaagaagcctggggcctcagtgaaggtttcctgcaaggcctctggatacaccttcactagttatgctatacattgggtgcgccaggcccccggacaaaggcttgagtggatggggtggatcaaggctggcaatggtaatacaagatattcacagaagttccaggacagagtcaccattaccagggacacatccacgaccacagcctacatggagctgagcagcctgagatctgaagacacggctgtgtattactgtgccctacttacggtgctaactcctgatgatgcttttgatatctggggccaggggaccatggtcaccgtctcttca

SEQ ID NO: 58 - DNA, 339 bp, homo sapiens
gacatcgtgatgacccagtctccagactccctggctgtgtctctgggcgagagggccaccatcaactgcaagtccagccagagtgttctatacagctccaacaataagaactacttagcttggtaccagcagaaaccaggacagcctcctaacctgctcatttactgggcatctacccggcaatccggggtccctgaccgattcagtggcagcgggtctgggacagatttcactctcaccatcagcagcctgcaggctgaagatgtggcagtttattactgtcaccagtattatagtagtcctctcactttcggcggagggaccaaggtggaaatcaaa

SEQ ID NO: 59 - DNA, 1353 bp, homo sapiens
caggtgcagcttgtgcagtctggggctgaggtgaagaagcctggggcctcagtgaaggtttcctgcaaggcctctggatacaccttcactagttatgctatacattgggtgcgccaggcccccggacaaaggcttgagtggatggggtggatcaaggctggcaatggtaatacaagatattcacagaagttccaggacagagtcaccattaccagggacacatccacgaccacagcctacatggagctgagcagcctgagatctgaagacacggctgtgtattactgtgccctacttacggtgctaactcctgatgatgcttttgatatctggggccaggggaccatggtcaccgtctcttcagcgtcgaccaagggcccatcggtcttccccctggcaccctcctccaagagcacctctgggggcacagcggccctgggctgcctggtcaaggactacttccccgaacccgtgacggtgtcgtggaactcaggcgccctgaccagcggcgtgcacaccttcccggctgtcctacagtcctcaggactctactccctcagcagcgtggtgaccgtgccctccagcagcttgggcacccagacctacatctgcaacgtgaatcacaagcccagcaacaccaaggtggacaagaaagttgagcccaaatcttgtgacaaaactcacacatgcccaccgtgcccagcacctgaactcctggggggaccgtcagtcttcctcttccccccaaaacccaaggacaccctcatgatctcccggacccctgaggtcacatgcgtggtggtggacgtgagccacgaagaccctgaggtcaagttcaactggtacgtggacggcgtggaggtgcataatgccaagacaaagccgcgggaggagcagtacaacagcacgtaccgtgtggtcagcgtcctcaccgtcctgcaccaggactggctgaatggcaaggagtacaagtgcaaggtctccaacaaagccctcccagcccccatcgagaaaaccatctccaaagccaaagggcagccccgagaaccacaggtgtacaccctgcccccatcccgggatgagctgaccaagaaccaggtcagcctgacctgcctggtcaaaggcttctatcccagcgacatcgccgtggagtgggagagcaatgggcagccggagaacaactacaagaccacgcctcccgtgctggactccgacggctccttcttcctctacagcaagctcaccgtggacaagagcaggtggcagcaggggaacgtcttctcatgctccgtgatgcatgaggctctgcacaaccactacacgcagaagagcctctccctgtctccgggtaaa

SEQ ID NO: 60 - DNA, 660 bp, homo sapiens
gacatcgtgatgacccagtctccagactccctggctgtgtctctgggcgagagggccaccatcaactgcaagtccagccagagtgttctatacagctccaacaataagaactacttagcttggtaccagcagaaaccaggacagcctcctaacctgctcatttactgggcatctacccggcaatccggggtccctgaccgattcagtggcagcgggtctgggacagatttcactctcaccatcagcagcctgcaggctgaagatgtggcagtttattactgtcaccagtattatagtagtcctctcactttcggcggagggaccaaggtggaaatcaaacgtacggtggctgcaccatctgtcttcatcttcccgccatctgatgagcagttgaaatctggaactgcctctgttgtgtgcctgctgaataacttctaccccagagaagccaaagtgcagtggaaggtggacaacgccctgcagagcggaaacagccaggaaagcgtgacagagcaggattccaaggattccacatacagcctgagcagcacactgacactgtccaaggccgactacgagaagcacaaggtgtacgcctgcgaagtgacacaccagggactgtcctcccctgtgacaaagagcttcaacagaggagaatgc

SEQ ID NO: 61 - protein, 15 aa, Artificial Sequence
  Synthetic peptide
PADGNPDPNANPNVD

SEQ ID NO: 62 - protein, 15 aa, Artificial Sequence
  Synthetic peptide
NPDPNANPNVDPNAN

SEQ ID NO: 63 - protein, 15 aa, Artificial Sequence
  Synthetic peptide
NANPNVDPNANPNVD

SEQ ID NO: 64 - protein, 15 aa, Artificial Sequence
  Synthetic peptide
NVDPNANPNVDPNAN

SEQ ID NO: 65 - protein, 15 aa, Artificial Sequence
  Synthetic peptide
NANPNVDPNANPNVD

SEQ ID NO: 66 - protein, 15 aa, Artificial Sequence
  Synthetic peptide
NVDPNANPNVDPNAN

SEQ ID NO: 67 - protein, 15 aa, Artificial Sequence
  Synthetic peptide
NANPNVDPNANPNAN

SEQ ID NO: 68 - protein, 15 aa, Artificial Sequence
  Synthetic peptide
NVDPNANPNANPNAN

SEQ ID NO: 69 - protein, 15 aa, Artificial Sequence
  Synthetic peptide
NANPNANPNANPNAN

SEQ ID NO: 70 - protein, 15 aa, Artificial Sequence
  Synthetic peptide
NANPNANPNANPNVD

SEQ ID NO: 71 - protein, 15 aa, Artificial Sequence
  Synthetic peptide
NANPNANPNVDPNAN

SEQ ID NO: 72 - protein, 15 aa, Artificial Sequence
  Synthetic peptide
NANPNVDPNANPNAN

SEQ ID NO: 73 - protein, 15 aa, Artificial Sequence
  Synthetic peptide
NVDPNANPNANPNAN

SEQ ID NO: 74 - protein, 15 aa, Artificial Sequence
  Synthetic peptide
NANPNANPNANPNKN

SEQ ID NO: 75 - protein, 15 aa, Artificial Sequence
  Synthetic peptide
NANPNANPNKNNQGN

SEQ ID NO: 76 - protein, 15 aa, Artificial Sequence
  Synthetic peptide
NANPNKNNQGNGQGH

SEQ ID NO: 77 - protein, 15 aa, Artificial Sequence
  Synthetic peptide
QEYQCYGSSSNTRVL

SEQ ID NO: 78 - protein, 15 aa, Artificial Sequence
  Synthetic peptide
KLKQPADGNPDPNAN

SEQ ID NO: 79 - protein, 36 aa, Artificial Sequence
  Synthetic peptide
NANPNANPNANPNANPNANPNANPNANPNANPNANP

SEQ ID NO: 80 - protein, 397 aa, plasmodium falciparum
MMRKLAILSVSSFLFVEALFQEYQCYGSSSNTRVLNELNYDNAGTNLYNELEMNYYGKQENWYSLKKNSRSLGENDDGNNEDNEKLRKPKHKKLKQPADGNPDPNANPNVDPNANPNVDPNANPNVDPNANPNANPNANPNANPNANPNANPNANPNANPNANPNANPNANPNANPNANPNANPNANPNANPNANPNVDPNANPNANPNANPNANPNANPNANPNANPNANPNANPNANPNANPNANPNANPNANPNANPNANPNANPNANPNKNNQGNGQGHNMPNDPNRNVDENANANSAVKNNNNEEPSDKHIKEYLNKIQNSLSTEWSPCSVTCGNGIQVRIKPGSANKPKDELDYANDIEKKICKMEKCSSVFNVVNSSIGLIMVLSFLFLN

SEQ ID NO: 81 - protein, 123 aa, homo sapiens
EVQLVESGGGVVQPGRSLRLSCEASGFTFSTYGMHWVRQAPGKGLEWVAIIWHDGSKKYHADSVRGRFTISRDNSKNTLYLQMNSLRAEDTAVYFCARVGNYGGDWGAGFDYWGQGTLVTVSS

SEQ ID NO: 82 - protein, 106 aa, homo sapiens
DIQMTQSPSFLSASVGDRVTIACRASQSISSWLAWYQQKPGKAPKLLIYHASSLESGVPSRFSGSASGTEFALTISSLQPDDFATYYCQQYSSYWTFGQGTKVEIK

SEQ ID NO: 83 - DNA, 369 bp, homo sapiens
gaggtacagctggtcgaaagcggagggggggtcgtacaaccagggcgatcattgcggttaagctgtgaggcctcgggattcacattctcaacctatggaatgcactgggtgagacaggcaccaggaaaggggcttgagtgggtggctattatttggcacgatggaagcaaaaagtatcacgctgacagcgtacgaggtcgctttacaatctcacgtgacaactccaaaaacacgctatatttgcaaatgaatagtctgcgtgcagaggatacagcagtctatttctgtgcacgagttgggaactacggaggcgactggggtgccgggtttgattactgggggcaagggacacttgttactgttagctct

SEQ ID NO: 84 - DNA, 318 bp, homo sapiens
gacatacaaatgacccaatcgccctcgttcctttcggcgagcgtcggtgatcgtgtcaccatagcctgccgggcaagtcaatcgatctcgagttggttggcgtggtatcagcagaaacctgggaaggctcccaaactattaatttatcacgcctcatctttagaatctggggtgccctcacgattttctggctcagcgagtggcactgagtttgccttaacaatcagctcattacaacctgatgactttgcaacatactactgtcaacagtacagctcttactggacatttgggcaggggaccaaagtcgaaattaac

SEQ ID NO: 85 - protein, 453 aa, homo sapiens
EVQLVESGGGVVQPGRSLRLSCEASGFTFSTYGMHWVRQAPGKGLEWVAIIWHDGSKKYHADSVRGRFTISRDNSKNTLYLQMNSLRAEDTAVYFCARVGNYGGDWGAGFDYWGQGTLVTVSSPSTKGPSVFPLAPSSKSTSGGTAALGCLVKDYFPEPVTVSWNSGALTSGVHTFPAVLQSSGLYSLSSVVTVPSSSLGTQTYICNVNHKPSNTKVDKKVEPKSCDKTHTCPPCPAPELLGGPSVFLFPPKPKDTLMISRTPEVTCVVVDVSHEDPEVKFNWYVDGVEVHNAKTKPREEQYNSTYRVVSVLTVLHQDWLNGKEYKCKVSNKALPAPIEKTISKAKGQPREPQVYTLPPSRDELTKNQVSLTCLVKGFYPSDIAVEWESNGQPENNYKTTPPVLDSDGSFFLYSKLTVDKSRWQQGNVFSCSVMHEALHNHYTQKSLSLSPGK

SEQ ID NO: 86 - DNA, 1359 bp, homo sapiens
gaggtacagctggtcgaaagcggagggggggtcgtacaaccagggcgatcattgcggttaagctgtgaggcctcgggattcacattctcaacctatggaatgcactgggtgagacaggcaccaggaaaggggcttgagtgggtggctattatttggcacgatggaagcaaaaagtatcacgctgacagcgtacgaggtcgctttacaatctcacgtgacaactccaaaaacacgctatatttgcaaatgaatagtctgcgtgcagaggatacagcagtctatttctgtgcacgagttgggaactacggaggcgactggggtgccgggtttgattactgggggcaagggacacttgttactgttagctctccgtcgaccaagggcccatcggtcttccccctggcaccctcctccaagagcacctctgggggcacagcggccctgggctgcctggtcaaggactacttccccgaaccggtgacggtgtcgtggaactcaggcgccctgaccagcggcgtgcacaccttcccggctgtcctacagtcctcaggactctactccctcagcagcgtggtgaccgtgccctccagcagcttgggcacccagacctacatctgcaacgtgaatcacaagcccagcaacaccaaggtggacaagaaagttgagcccaaatcttgtgacaaaactcacacatgcccaccgtgcccagcacctgaactcctggggggaccgtcagtcttcctcttccccccaaaacccaaggacaccctcatgatctcccggacccctgaggtcacatgcgtggtggtggacgtgagccacgaagaccctgaggtcaagttcaactggtacgtggacggcgtggaggtgcataatgccaagacaaagccgcgggaggagcagtacaacagcacgtaccgtgtggtcagcgtcctcaccgtcctgcaccaggactggctgaatggcaaggagtacaagtgcaaggtctccaacaaagccctcccagcccccatcgagaaaaccatctccaaagccaaagggcagccccgagaaccacaggtgtacaccctgcccccatcccgggatgagctgaccaagaaccaggtcagcctgacctgcctggtcaaaggcttctatcccagcgacatcgccgtggagtgggagagcaatgggcagccggagaacaactacaagaccacgcctcccgtgctggactccgacggctccttcttcctctacagcaagctcaccgtggacaagagcaggtggcagcaggggaacgtcttctcatgctccgtgatgcatgaggctctgcacaaccactacacgcagaagagcctctccctgtctccgggtaaa

SEQ ID NO: 87 - protein, 213 aa, homo sapiens
DIQMTQSPSFLSASVGDRVTIACRASQSISSWLAWYQQKPGKAPKLLIYHASSLESGVPSRFSGSASGTEFALTISSLQPDDFATYYCQQYSSYWTFGQGTKVEIKRTVAAPSVFIFPPSDEQLKSGTASVVCLLNNFYPREAKVQWKVDNALQSGNSQESVTEQDSKDSTYSLSSTLTLSKADYEKHKVYACEVTHQGLSSPVTKSFNRGEC

SEQ ID NO: 88 - protein, 4 aa, homo sapiens
YGMH

SEQ ID NO: 89 - protein, 17 aa, homo sapiens
IIWHDGSKKYHADSVRG

SEQ ID NO: 90 - protein, 15 aa, homo sapiens
RVGNYGGDWGAGFDY

SEQ ID NO: 91 - protein, 11 aa, homo sapiens
RASQSISSWLA

SEQ ID NO: 92 - protein, 7 aa, homo sapiens
HASSLES

SEQ ID NO: 93 - protein, 8 aa, homo sapiens
QQYSSYWT

SEQ ID NO: 94 - protein, 15 aa, Artificial Sequence
  Synthetic peptide
APDPNANPNVDPNAN

SEQ ID NO: 95 - protein, 15 aa, Artificial Sequence
  Synthetic peptide
NADPNANPNVDPNAN

SEQ ID NO: 96 - protein, 15 aa, Artificial Sequence
  Synthetic peptide
NPAPNANPNVDPNAN

SEQ ID NO: 97 - protein, 15 aa, Artificial Sequence
  Synthetic peptide
NPDANANPNVDPNAN

SEQ ID NO: 98 - protein, 15 aa, Artificial Sequence
  Synthetic peptide
NPDPAANPNVDPNAN

SEQ ID NO: 99 - protein, 15 aa, Artificial Sequence
  Synthetic peptide
NPDPNSNPNVDPNAN

SEQ ID NO: 100 - protein, 15 aa, Artificial Sequence
  Synthetic peptide
NPDPNAAPNVDPNAN

SEQ ID NO: 101 - protein, 15 aa, Artificial Sequence
  Synthetic peptide
NPDPNANANVDPNAN

SEQ ID NO: 102 - protein, 15 aa, Artificial Sequence
  Synthetic peptide
NPDPNANPAVDPNAN

SEQ ID NO: 103 - protein, 15 aa, Artificial Sequence
  Synthetic peptide
NPDPNANPNADPNAN

SEQ ID NO: 104 - protein, 15 aa, Artificial Sequence
  Synthetic peptide
NPDPNANPNVAPNAN

SEQ ID NO: 105 - protein, 15 aa, Artificial Sequence
  Synthetic peptide
NPDPNANPNVDANAN

SEQ ID NO: 106 - protein, 15 aa, Artificial Sequence
  Synthetic peptide
NPDPNANPNVDPAAN

SEQ ID NO: 107 - protein, 15 aa, Artificial Sequence
  Synthetic peptide
NPDPNANPNVDPNSN

SEQ ID NO: 108 - protein, 15 aa, Artificial Sequence
  Synthetic peptide
NPDPNANPNVDPNRN

SEQ ID NO: 109 - protein, 15 aa, Artificial Sequence
  Synthetic peptide
NPDPNANPNVDPNAA

SEQ ID NO: 110 - protein, 15 aa, Artificial Sequence
  Synthetic peptide
NPDPNGNPNVDPNAN

SEQ ID NO: 111 - protein, 15 aa, Artificial Sequence
  Synthetic peptide
NPDPNVNPNVDPNAN

SEQ ID NO: 112 - protein, 15 aa, Artificial Sequence
  Synthetic peptide
NPDPNPNPNVDPNAN

SEQ ID NO: 113 - protein, 15 aa, Artificial Sequence
  Synthetic peptide
NPDPNAAPNVDPNAN

SEQ ID NO: 114 - protein, 15 aa, Artificial Sequence
  Synthetic peptide
NPDPNANANVDPNAN

SEQ ID NO: 115 - protein, 15 aa, Artificial Sequence
  Synthetic peptide
NPDPNANPAVDPNAN

SEQ ID NO: 116 - protein, 15 aa, Artificial Sequence
  Synthetic peptide
NPDPNANPAVDPAAN

SEQ ID NO: 117 - protein, 121 aa, Artificial Sequence
  Synthetic peptide
QVQLVQSGAEVKKPGASVKVSCKASGYTFTSYAIHWVRQAPGQRLEWMGWIKAGNGGGGYSGKFQDRVTITRDTSTTTAYMELSSLRSEDTAVYYCALLTVLTPDDAFDIWGQGTMVTVSS

SEQ ID NO: 118 - protein, 19 aa, Artificial Sequence
  Synthetic peptide
MGWSCIILFLVATATGVHS

SEQ ID NO: 119 - protein, 454 aa, homo sapiens
QVQLVESGGGVVQPGRSLRLSCAASGFTFSSYGIHWVRQAPGKGLEWVAVIWYDGSKKYYGDSVKGRFTISRDNSKNTLYLQMNSLRVEDTAVYYCARAVIAATGTRGYWFDPWGQGTLVTVSSASTKGPSVFPLAPSSKSTSGGTAALGCLVKDYFPEPVTVSWNSGALTSGVHTFPAVLQSSGLYSLSSVVTVPSSSLGTQTYICNVNHKPSNTKVDKKVEPKSCDKTHTCPPCPAPELLGGPSVFLFPPKPKDTLMISRTPEVTCVVVDVSHEDPEVKFNWYVDGVEVHNAKTKPREEQYNSTYRVVSVLTVLHQDWLNGKEYKCKVSNKALPAPIEKTISKAKGQPREPQVYTLPPSRDELTKNQVSLTCLVKGFYPSDIAVEWESNGQPENNYKTTPPVLDSDGSFFLYSKLTVDKSRWQQGNVFSCSVMHEALHNHYTQKSLSLSPGK

SEQ ID NO: 120 - protein, 213 aa, homo sapiens
DIIMTQSPVSLSASVGDRVTITCRASQSISSHLNWYQQKPGKAPKLLIYAASSLQSGVPSRFSGSGSGTDFTLTISSLQPEDFATYSCQQTYRGFTFAPGTKVDIKRTVAAPSVFIFPPSDEQLKSGTASVVCLLNNFYPREAKVQWKVDNALQSGNSQESVTEQDSKDSTYSLSSTLTLSKADYEKHKVYACEVTHQGLSSPVTKSFNRGEC

SEQ ID NO: 121 - DNA, 1362 bp, Artificial sequence
  anitbody heavy chain
caggtgcagctggtggagtctgggggaggcgtggtccagcctgggaggtccctgagactctcctgtgcagcgtctggattcaccttcagtagctatggcatacactgggtccgccaggctccaggcaaggggctggagtgggtggcagttatatggtatgatggaagtaagaaatattatggagactctgtgaagggccgattcaccatctccagagacaattccaagaacacgctgtatctgcaaatgaacagcctgagagtcgaggacacggctgtgtattactgtgcgagggctgttatagcagcaactggtacgcgaggttactggttcgacccctggggccagggaaccctggtcaccgtctcctcagcgtcgaccaagggcccatcggtcttccccctggcaccctcctccaagagcacctctgggggcacagcggccctgggctgcctggtcaaggactacttccccgaacccgtgacggtgtcgtggaactcaggcgccctgaccagcggcgtgcacaccttcccggctgtcctacagtcctcaggactctactccctcagcagcgtggtgaccgtgccctccagcagcttgggcacccagacctacatctgcaacgtgaatcacaagcccagcaacaccaaggtggacaagaaagttgagcccaaatcttgtgacaaaactcacacatgcccaccgtgcccagcacctgaactcctggggggaccgtcagtcttcctcttccccccaaaacccaaggacaccctcatgatctcccggacccctgaggtcacatgcgtggtggtggacgtgagccacgaagaccctgaggtcaagttcaactggtacgtggacggcgtggaggtgcataatgccaagacaaagccgcgggaggagcagtacaacagcacgtaccgtgtggtcagcgtcctcaccgtcctgcaccaggactggctgaatggcaaggagtacaagtgcaaggtctccaacaaagccctcccagcccccatcgagaaaaccatctccaaagccaaagggcagccccgagaaccacaggtgtacaccctgcccccatcccgggatgagctgaccaagaaccaggtcagcctgacctgcctggtcaaaggcttctatcccagcgacatcgccgtggagtgggagagcaatgggcagccggagaacaactacaagaccacgcctcccgtgctggactccgacggctccttcttcctctacagcaagctcaccgtggacaagagcaggtggcagcaggggaacgtcttctcatgctccgtgatgcatgaggctctgcacaaccactacacgcagaagagcctctccctgtctccgggtaaa

SEQ ID NO: 122 - DNA, 639 bp, artificial sequence
  antibody light chain
gacatcattatgacccagtctccagtctccctgtctgcatctgtaggagacagagtcaccatcacttgccgggcaagtcagagcattagcagccatttaaattggtatcagcagaaaccagggaaagcccctaagctcctgatctatgctgcatccagtttgcaaagtggggtcccatcaaggttcagtggcagtggatctgggacagatttcactctcaccatcagcagtctgcaacctgaagattttgcaacttactcctgtcaacagacttacagggggttcactttcgcccctgggaccaaagtggatatcaaacgtacggtggctgcaccatctgtcttcatcttcccgccatctgatgagcagttgaaatctggaactgcctctgttgtgtgcctgctgaataacttctaccccagagaagccaaagtgcagtggaaggtggacaacgccctgcagagcggaaacagccaggaaagcgtgacagagcaggattccaaggattccacatacagcctgagcagcacactgacactgtccaaggccgactacgagaagcacaaggtgtacgcctgcgaagtgacacaccagggactgtcctcccctgtgacaaagagcttcaacagaggagaatgc

SEQ ID NO: 123 - DNA, 369 bp, artificial sequence
  codon-optimized antibody heavy chain
gaggtgcagctggtggaaagcggcggaggcgtggtgcagcctggcagatctctgagactgagctgcgaggccagcggcttcaccttcagcacctacggcatgcactgggtgcgccaggcccctggaaaaggcctggaatgggtggccatcatctggcacgacggcagcaagaagtaccacgccgatagcgtgcggggcagattcaccatcagccgggacaacagcaagaacaccctgtacctgcagatgaacagcctgcgggccgaggataccgccgtgtacttctgtgccagagtgggcaactacggcggcgattggggagccggctttgactattggggccagggcacactcgtgaccgtgtcctct

SEQ ID NO: 124 - DNA, 318 bp, artificial sequence
  codon-optimized antibody light chain
gacatccagatgacccagagccccagcttcctgagcgccagcgtgggcgacagagtgacaatcgcctgtagagccagccagagcatcagcagctggctggcctggtatcagcagaagcctggcaaggcccccaaactgctgatctaccacgccagcagcctggaaagcggcgtgcccagcagattttctggcagcgcctccggcaccgagttcgccctgacaatcagctccctgcagcccgacgacttcgccacctactactgccagcagtacagcagctactggaccttcggccagggcaccaaggtggaaatcaag